European Patent Application EP 4 368 629 A1, published May 15, 2024. Title: PEPTIDE AND COMPOSITION. Applicant: Oasaka University. Application EP 22837707.3, filed July 6, 2022. The sequence listing filed with the application follows.

SEQUENCE LISTING (101 sequences)

SEQ ID NO: 1 - protein, 9 aa, synthetic construct
TQAERSIIG

SEQ ID NO: 2 - protein, 9 aa, synthetic construct
ERSIIGMID

SEQ ID NO: 3 - protein, 9 aa, synthetic construct
IIGMIDMFH

SEQ ID NO: 4 - protein, 9 aa, synthetic construct
MIDMFHKYT

SEQ ID NO: 5 - protein, 9 aa, synthetic construct
RRDDKIEKP

SEQ ID NO: 6 - protein, 9 aa, synthetic construct
DKIEKPSLL

SEQ ID NO: 7 - protein, 9 aa, synthetic construct
EKPSLLTMM

SEQ ID NO: 8 - protein, 9 aa, synthetic construct
SLLTMMKEN

SEQ ID NO: 9 - protein, 9 aa, synthetic construct
TMMKENFPN

SEQ ID NO: 10 - protein, 9 aa, synthetic construct
MKENFPNFL

SEQ ID NO: 11 - protein, 9 aa, synthetic construct
FEKKDKNED

SEQ ID NO: 12 - protein, 9 aa, synthetic construct
KDKNEDKKI

SEQ ID NO: 13 - protein, 9 aa, synthetic construct
NEDKKIDFS

SEQ ID NO: 14 - protein, 9 aa, synthetic construct
KKIDFSEFL

SEQ ID NO: 15 - protein, 9 aa, synthetic construct
DFSEFLSLL

SEQ ID NO: 16 - protein, 9 aa, synthetic construct
EFLSLLGDI

SEQ ID NO: 17 - protein, 9 aa, synthetic construct
SLLGDIATD

SEQ ID NO: 18 - protein, 9 aa, synthetic construct
GDIATDYHK

SEQ ID NO: 19 - protein, 9 aa, synthetic construct
ATDYHKQSH

SEQ ID NO: 20 - protein, 9 aa, synthetic construct
TELEKALNS

SEQ ID NO: 21 - protein, 9 aa, synthetic construct
EKALNSIID

SEQ ID NO: 22 - protein, 9 aa, synthetic construct
LNSIIDVYH

SEQ ID NO: 23 - protein, 9 aa, synthetic construct
IIDVYHKYS

SEQ ID NO: 24 - protein, 9 aa, synthetic construct
GNFHAVYRD

SEQ ID NO: 25 - protein, 9 aa, synthetic construct
HAVYRDDLK

SEQ ID NO: 26 - protein, 9 aa, synthetic construct
YRDDLKKLL

SEQ ID NO: 27 - protein, 9 aa, synthetic construct
DLKKLLETE

SEQ ID NO: 28 - protein, 9 aa, synthetic construct
KLLETECPQ

SEQ ID NO: 29 - protein, 9 aa, synthetic construct
LETECPQYI

SEQ ID NO: 30 - protein, 9 aa, synthetic construct
FKELDINTD

SEQ ID NO: 31 - protein, 9 aa, synthetic construct
LDINTDGAV

SEQ ID NO: 32 - protein, 9 aa, synthetic construct
NTDGAVNFQ

SEQ ID NO: 33 - protein, 9 aa, synthetic construct
GAVNFQEFL

SEQ ID NO: 34 - protein, 9 aa, synthetic construct
NFQEFLILV

SEQ ID NO: 35 - protein, 9 aa, synthetic construct
EFLILVIKM

SEQ ID NO: 36 - protein, 9 aa, synthetic construct
ILVIKMGVA

SEQ ID NO: 37 - protein, 9 aa, synthetic construct
IKMGVAAHK

SEQ ID NO: 38 - protein, 9 aa, synthetic construct
GVAAHKKSH

SEQ ID NO: 39 - protein, 9 aa, synthetic construct
SQLERNIET

SEQ ID NO: 40 - protein, 9 aa, synthetic construct
ERNIETIIN

SEQ ID NO: 41 - protein, 9 aa, synthetic construct
IETIINTFH

SEQ ID NO: 42 - protein, 9 aa, synthetic construct
IINTFHQYS

SEQ ID NO: 43 - protein, 9 aa, synthetic construct
GHPDTLNQG

SEQ ID NO: 44 - protein, 9 aa, synthetic construct
DTLNQGEFK

SEQ ID NO: 45 - protein, 9 aa, synthetic construct
NQGEFKELV

SEQ ID NO: 46 - protein, 9 aa, synthetic construct
EFKELVRKD

SEQ ID NO: 47 - protein, 9 aa, synthetic construct
ELVRKDLQN

SEQ ID NO: 48 - protein, 9 aa, synthetic construct
VRKDLQNFL

SEQ ID NO: 49 - protein, 9 aa, synthetic construct
MEDLDTNAD

SEQ ID NO: 50 - protein, 9 aa, synthetic construct
LDTNADKQL

SEQ ID NO: 51 - protein, 9 aa, synthetic construct
NADKQLSFE

SEQ ID NO: 52 - protein, 9 aa, synthetic construct
KQLSFEEFI

SEQ ID NO: 53 - protein, 9 aa, synthetic construct
SFEEFIMLM

SEQ ID NO: 54 - protein, 9 aa, synthetic construct
EFIMLMARL

SEQ ID NO: 55 - protein, 9 aa, synthetic construct
MLMARLTWA

SEQ ID NO: 56 - protein, 9 aa, synthetic construct
ARLTWASHE

SEQ ID NO: 57 - protein, 9 aa, synthetic construct
TWASHEKMH

SEQ ID NO: 58 - protein, 9 aa, synthetic construct
PDTLNQGEF

SEQ ID NO: 59 - protein, 9 aa, synthetic construct
KHHAKVGSA

SEQ ID NO: 60 - protein, 9 aa, synthetic construct
TLVNSVNSK

SEQ ID NO: 61 - protein, 101 aa, Pteropus alecto
MSHTQAEKAVMDMIELFHTYTKPDDMIDEPGLTKMLQENFPTFLSACGKKGKDYLSHIFEDKDQNKDKKIEFSEFLSVIGDIATDYHKQSHGAPACSGGSQ

SEQ ID NO: 62 - protein, 101 aa, Myotis davidii
MSHTPVEQSVEDLIVLFHKYTKPDDKIDKPGLLKMLKENFPNFLKACEKKGKDFLAHIFEDEDKNKDKKIDFSEFLLVLGVIATDYHNHSHGAPLCSGGGH

SEQ ID NO: 63 - protein, 101 aa, Ursus maritimus
MSSTRAEKFMVGILELFHNDTRHHDTTDKPALLKTLQEDFPKFLSACDKKGTAYWANIFEKKGKNGDKKIEFSKFLSLLGEITMDFHKQSHGAASCSTGSQ

SEQ ID NO: 64 - protein, 101 aa, Equus caballus
MSETEAEASVIGIIELFHKYTGRDDMIDKPGLLKMLQDNFPNFLAACDKKGTDYLANVFEKKDKNRDKKIDFSEFLSLLGDIATDYHKQSHGAPACSEGDQ

SEQ ID NO: 65 - protein, 101 aa, Tupaia chinensis
MSNTQAEESIVGMIDLFHKYTGRDDAIDKPSLLKMMKENFPNFLSACEHKGTDYLANVFEKKDKNKDKKIEFSEFLSMMGDIATDYHKQSHGASACSGKSH

SEQ ID NO: 66 - protein, 101 aa, Homo sapiens
MSNTQAERSIIGMIDMFHKYTRRDDKIEKPSLLTMMKENFPNFLSACDKKGTNYLADVFEKKDKNEDKKIDFSEFLSLLGDIATDYHKQSHGAAPCSGGSQ

SEQ ID NO: 67 - protein, 101 aa, Myotis brandtii
MSHTHAEKYVMTMIDLFHKYSKPDDMIDQPGLLMLLKENFPNFVKGCDRRGNNYLSQVFEEKDLNEDKKIQFSEFLCLLGDIAMDYHRQSHGAAPCSGGRQ

SEQ ID NO: 68 - protein, 101 aa, Bos taurus
MSSSQLEQAITDLINLFHKYSGSDDTIEKEDLLRLMKDNFPNFLGACEKRGRDYLSNIFEKQDKNKDRKIDFSEFLSLLADIATDYHNHSHGAQLCSGGNQ

SEQ ID NO: 69 - protein, 93 aa, Homo sapiens
MLTELEKALNSIIDVYHKYSLIKGNFHAVYRDDLKKLLETECPQYIRKKGADVWFKELDINTDGAVNFQEFLILVIKMGVAAHKKSHEESHKE

SEQ ID NO: 70 - protein, 89 aa, Bos taurus
MLTDLECAINSLIDVYHKYSLKKGNYHAVYRDDLKQLLETECPKFMKKKDADTWFKELDINQDGGINFEEFLVLVIKVGLEAHEEIHKE

SEQ ID NO: 71 - protein, 89 aa, Mus musculus
MPSELEKALSNLIDVYHNYSNIQGNHHALYKNDFKKMVTTECPQFVQNINIENLFRELDINSDNAINFEEFLAMVIKVGVASHKDSHKE

SEQ ID NO: 72 - protein, 89 aa, Rattus norvegicus
MATELEKALSNVIEVYHNYSGIKGNHHALYRDDFRKMVTTECPQFVQNKNTESLFKELDVNSDNAINFEEFLVLVIRVGVAAHKDSHKE

SEQ ID NO: 73 - protein, 114 aa, Homo sapiens
MTCKMSQLERNIETIINTFHQYSVKLGHPDTLNQGEFKELVRKDLQNFLKKENKNEKVIEHIMEDLDTNADKQLSFEEFIMLMARLTWASHEKMHEGDEGPGHHHKPGLGEGTP

SEQ ID NO: 74 - protein, 156 aa, Bos sp.
MEDKMSQMESSIETIINIFHQYSVRLGHYDTLIQKEFKQLVQKELPNFLKKQKKNEAAINEIMEDLDTNVDKQLSFEEFIMLVARLTVASHEEMHNTAPPGQGHRHGPGYGKGGSGSCSGQGSPDQGSHDLGSHGHGHGHSHGGHGHSHGGHGHSH

SEQ ID NO: 75 - protein, 132 aa, Oryctolagus cuniculus
MSCGMSQLERSIDTIINVFHQYSVRVGPRDSLSQKEFKQLVQKELHNFLKKEARDEKAINDIMEDLDTNQDKQLSFEEFVILMARLVHASHEEMHKNAPHDHEGHSHGPGLGGGGPGHGHGHSHGHGHGHSH

SEQ ID NO: 76 - protein, 113 aa, Mus musculus
MANKAPSQMERSITTIIDTFHQYSRKEGHPDTLSKKEFRQMVEAQLATFMKKEKRNEALINDIMEDLDTNQDNQLSFEECMMLMAKLIFACHEKLHENNPRGHGHSHGKGCGK

SEQ ID NO: 77 - protein, 113 aa, Rattus norvegicus
MAAKTGSQLERSISTIINVFHQYSRKYGHPDTLNKAEFKEMVNKDLPNFLKREKRNENLLRDIMEDLDTNQDNQLSFEECMMLMGKLIFACHEKLHENNPRGHDHSHGKGCGK

SEQ ID NO: 78 - protein, 18 aa, synthetic construct
TQAERSIIGMIDMFHKYT

SEQ ID NO: 79 - protein, 9 aa, synthetic construct
TQAERSIIG

SEQ ID NO: 80 - protein, 9 aa, synthetic construct
ERSIIGMID

SEQ ID NO: 81 - protein, 9 aa, synthetic construct
IIGMIDMFH

SEQ ID NO: 82 - protein, 9 aa, synthetic construct
MIDMFHKYT

SEQ ID NO: 83 - protein, 94 aa, Pteropus alecto
MSHTQAEKAVMDMIELFHTYTKPDDMIDEPGLTKMLQENFPTFLSACGKKGKDYLSHIFEDKDQNKDKKIEFSEFLSVIGDIATDYHKQSHGAP

SEQ ID NO: 84 - protein, 94 aa, Myotis davidii
MSHTPVEQSVEDLIVLFHKYTKPDDKIDKPGLLKMLKENFPNFLKACEKKGKDFLAHIFEDEDKNKDKKIDFSEFLLVLGVIATDYHNHSHGAP

SEQ ID NO: 85 - protein, 94 aa, Ursus maritimus
MSSTRAEKFMVGILELFHNDTRHHDTTDKPALLKTLQEDFPKFLSACDKKGTAYWANIFEKKGKNGDKKIEFSKFLSLLGEITMDFHKQSHGAA

SEQ ID NO: 86 - protein, 94 aa, Equus caballus
MSETEAEASVIGIIELFHKYTGRDDMIDKPGLLKMLQDNFPNFLAACDKKGTDYLANVFEKKDKNRDKKIDFSEFLSLLGDIATDYHKQSHGAP

SEQ ID NO: 87 - protein, 94 aa, Tupaia chinensis
MSNTQAEESIVGMIDLFHKYTGRDDAIDKPSLLKMMKENFPNFLSACEHKGTDYLANVFEKKDKNKDKKIEFSEFLSMMGDIATDYHKQSHGAS

SEQ ID NO: 88 - protein, 94 aa, Homo sapiens
MSNTQAERSIIGMIDMFHKYTRRDDKIEKPSLLTMMKENFPNFLSACDKKGTNYLADVFEKKDKNEDKKIDFSEFLSLLGDIATDYHKQSHGAA

SEQ ID NO: 89 - protein, 94 aa, Myotis brandtii
MSHTHAEKYVMTMIDLFHKYSKPDDMIDQPGLLMLLKENFPNFVKGCDRRGNNYLSQVFEEKDLNEDKKIQFSEFLCLLGDIAMDYHRQSHGAA

SEQ ID NO: 90 - protein, 94 aa, Bos taurus
MSSSQLEQAITDLINLFHKYSGSDDTIEKEDLLRLMKDNFPNFLGACEKRGRDYLSNIFEKQDKNKDRKIDFSEFLSLLADIATDYHNHSHGAQ

SEQ ID NO: 91 - protein, 90 aa, Homo sapiens
MLTELEKALNSIIDVYHKYSLIKGNFHAVYRDDLKKLLETECPQYIRKKGADVWFKELDINTDGAVNFQEFLILVIKMGVAAHKKSHEES

SEQ ID NO: 92 - protein, 89 aa, Bos taurus; identical to SEQ ID NO: 70

SEQ ID NO: 93 - protein, 89 aa, Mus musculus; identical to SEQ ID NO: 71

SEQ ID NO: 94 - protein, 89 aa, Rattus norvegicus; identical to SEQ ID NO: 72

SEQ ID NO: 95 - protein, 97 aa, Homo sapiens
MTCKMSQLERNIETIINTFHQYSVKLGHPDTLNQGEFKELVRKDLQNFLKKENKNEKVIEHIMEDLDTNADKQLSFEEFIMLMARLTWASHEKMHEG

SEQ ID NO: 96 - protein, 97 aa, Bos taurus
MEDKMSQMESSIETIINIFHQYSVRLGHYDTLIQKEFKQLVQKELPNFLKKQKKNEAAINEIMEDLDTNVDKQLSFEEFIMLVARLTVASHEEMHNT

SEQ ID NO: 97 - protein, 98 aa, Oryctolagus cuniculus
MSCGMSQLERSIDTIINVFHQYSVRVGPRDSLSQKEFKQLVQKELHNFLKKEARDEKAINDIMEDLDTNQDKQLSFEEFVILMARLVHASHEEMHKNA

SEQ ID NO: 98 - protein, 98 aa, Mus musculus
MANKAPSQMERSITTIIDTFHQYSRKEGHPDTLSKKEFRQMVEAQLATFMKKEKRNEALINDIMEDLDTNQDNQLSFEECMMLMAKLIFACHEKLHEN

SEQ ID NO: 99 - protein, 98 aa, Rattus norvegicus
MAAKTGSQLERSISTIINVFHQYSRKYGHPDTLNKAEFKEMVNKDLPNFLKREKRNENLLRDIMEDLDTNQDNQLSFEECMMLMGKLIFACHEKLHEN

SEQ ID NO: 100 - protein, 10 aa, synthetic construct
KLLETECPQY

SEQ ID NO: 101 - protein, 11 aa, synthetic construct
KLLETECPQYI